European Patent Application EP 4 541 881 A1, published April 23, 2025. Title: 治疗糖尿病及相关病症的两歧双歧杆菌. Applicant: 合肥瀚微生物科技有限公司. Application CN. The sequence listing filed with the application follows.

SEQUENCE LISTING (5 sequences)

SEQ ID NO: 1 - DNA, 1029 bp, Bifidobacterium bifidum
  source 1..1029: mol_type = genomic DNA
gacgccgcgtgagggatggaggccttcgggttgtaaacctcttttgtttgggagcaagccttcgggtgagtgtacctttcgaataagcgccggctaactacgtgccagcagccgcggtaatacgtagggcgcaagcgttatccggatttattgggcgtaaagggctcgtaggcggctcgtcgcgtccggtgtgaaagtccatcgcttaacggtggatctgcgccgggtacgggcgggctggagtgcggtaggggagactggaattcccggtgtaacggtggaatgtgtagatatcgggaagaacaccgatggcgaaggcaggtctctgggccgtcactgacgctgaggagcgaaagcgtggggagcgaacaggattagataccctggtagtccacgccgtaaacggtggacgctggatgtggggcacgttccacgtgttccgtgtcggagctaacgcgttaagcgtcccgcctggggagtacggccgcaaggctaaaactcaaagaaattgacgggggcccgcacaagcggcggagcatgcggattaattcgatgcaacgcgaagaaccttacctgggcttgacatgttcccgacgacgccagagatggcgtttcccttcggggcgggttcacaggtggtgcatggtcgtcgtcagctcgtgtcgtgagatgttgggttaagtcccgcaacgagcgcaaccctcgccccgtgttgccagcacgttatggtgggaactcacgggggaccgccggggttaactcggaggaaggtggggatgacgtcagatcatcatgccccttacgtccagggcttcacgcatgctacaatggccggtacagcgggatgcgacatggcgacatggagcggatccctgaaaaccggtctcagttcggatcggagcctgcaacccggctccgtgaaggcggagtcgctagtaatcgcggatcagcaacgccgcggtgaatgcgttcccgggccttgtacacaccgcccgtcaagtcatgaaagtgggcagcacccgaagccgg

SEQ ID NO: 2 - DNA, 6061 bp, Bifidobacterium bifidum
  source 1..6061: mol_type = genomic DNA
gattttgaaaaaagtctgcggcttttctttttgcccaaacgcagaaaggaggcgacggcctatgtacttcacttccggcagcgaccgggcctttgaacagctcatgcagggcaagcccggtttcgaccactacgacagcggcgaggcggtcacgccggaggactgcggcacctgccgcttttatcgcccgcactggaaatatcaattctgcgtctatgcggaatgtccctaccagccgggcaagctgaccgcctacgacgcggtgacatttcgagtgaaaggagttgagaacatggcagtatttcgtgtagagcgtaacaagggctacacggtgatgtccaatcaccacctgcggaacaaggacttatccctgaaagccaagggcctgttatcgcaaatgctctctctgccggaagattgggactatacgctcaaaggcttatcccttatcaaccgggagcagatcgacgcgatccgggccgcaatccgggagctggaacaggccgggtacatcgtccgatcccgtgagcgcgacagccaagggcgcttgcgcggcgcggactatgtgatctatgaacagccccaacctgtgccggattcacctacgttggaaaatccaatgttggataatccaacgcaggaaaagcctacgttgggaaaaccaacgcaattaaataaagatatatcaagtaaagaaaaaccaattactgatgtatcaattaccgatcccattcctatcctttcccgaccctctcctttggtggacgaggcggcacagccgccggaacggaaaggaacggaagcgaaatcacagagcgccatagagatttatcgtcaaatcatcatggacaacatcgagtacgaacacctttgccagcacgtcaagggcattgaccgggaaacgctggacgagattgtggacttgctggtggaaaccgtatgcagcgcccgcaagaccatccgcattgccggggacgattacccggcagagctggtgaaatccaagtttatgaagctggacagctctcacatcgagtttgtctttgactgtttgagcaaaaacacttcggaaattcgcaatatcaagaaatacctgctggctatgctgttcaatgcgcccagcacgatcaacggttactatgccgcgctcgtggcccatgacatgaacaccggcaaaatctgaaaggaggacggccctatgaaacagggtgcattgattttcgacgagcgcagcgaccgttacgatattcgctttgatctggcggactactacggcggcctgcactgtggagaaacctttgacgtgatggtgggcggcaggtggaagcccacccgcattgagtacggtgccaactggtatctggttggcatccgtgccgacgacctttccggcctgcgggtgaggatttaatcggggacaaccggcgcaagcggctgtcccttttctgtttcctgcggcggctgacggtgccaccttaaccgtgccgccgcacttctgcgaaaggagggatagcgattgcaggaggaagtaacccaaaagacaatagccttttccatcaaatcggccaagctgacaatccaagtgctgcaagcggcggcccgcaagtttctggaaacccaaaacaagggcaagaccaagctgcaccacggccagcagagcctaaagcagctcaaaaagcacggggcggccctgtccaatatcgagatcaccgacgccaacattggactgtttaagccctgtgccaagaaatacggcgtggacttcacgctgcggaaagacgccactacccagcccccgcactacattgtgatttttaaggccaaggacgccgacaacatggaacaggcgttcaaggagttcacggccaagaagttgcagcgggaggaacggccctcgatccgcaaggacattgccgcaagcaaggaaaaggcagcggcccgcaacgctgaccgggccaaggaaaaattcaaagaaagggggctgtcacgatgaagccggaaatgaaaaaactgataatcgccaatctgccctatctgctgtttgtctatctgttcggcaagctggggcaggcgtaccggctggcggagggcatcgacctttcccaaaagctcctgcactttgcggacggctgcgcggcggcctttgaaagtgctgcccccagcttccacctctttgacctgctgatcggcgtcgccggtgctgcggcgctgcggctcatggtgtactgcaaaggcaagaacgccaagaaataccgcaaaggcgtggagtacggcagcgcccgatggggcggccccaaggatatagccccctatatcgaccccaattttgacaacaacattctgctgacacagacggaacggctgacgatgaacaacaggccgaaagaccccaagaccgcacgaaacaagaatgtccttgtaatcggcggttccggctccggcaagacccggttctttgtaaaaccgaacctgatgcaatgtgtgtccaaggactatccgacttctttcgtgataaccgatcccaagggcagcttgatcggtgaagtgggccagctccttatccgcagcggctaccgcgtgaaagtgctgaacaccatcaatttttccaagagcatgaaatacaacccgtttcggtatctgcactcggaaaaagatgtgttgaagctggtaaacaccctgatttgcaacactaaaggtgagggcgaaaaaagcgcggaagatttttgggtgaaatcggaacggctgttctacacggccctgatcggctatatctggcaggaagcgccggaggaagaaatgaacttcacgacgctgcttgaaatgataaatgccagcgaagcccgcgaggacgacccggaatttcaatcgccggtggatttgatgtttgagcgattggaggaacgtgatccagaccactttgccgtccggcagtataaaaaattcctgctttcggcgggcaagacccgttcctcaatccttatcagcgcaggcgcgagaatggccccatttgacatccgcgaggtgcgggagctgatggaggacgacgaactggaacttgacaccatcggggacgagaaaacggcgctgttcctgattatgtcggacacggacaccacctttaatttcattctggcaatggtacagagccagcttatcaacctgctttgtgaccgggccgatgataaatacggcgggcggctgcctgttcacgtccgcatgattctggacgagtttgcgaacatcggccagatacccaactttgacaagttgatcgccaccatccgaagccgtgaaatctcggcttctattattttgcaaagccagtcacagttaaaggccatctacaaggacgctgcggaaatcatttccgacaactgcgactgtacgcttttccttagtgggcggggcaagaacgccaaggaaatctctgacgtgctgggcaaagaaaccatcgacagctacaaccagagcgaaaaccggggcgcacagacctctcacggattgaattatcagaaattaggaaaggagttgatgtcacaggacgagatcgcaacgatggacggaggcaagtgtattttgcaggtgcgcggtgtaaggccgtttttcagtgagaaatacgacattacccgtcacccccgctataaatacctttccgacgccgacaagaaaaactattttgacgtggacaggtacttgaccgccctgcgccggaaacggcagcgggtggtttcgcaggaggaaacctttgacctctacgacatagacctgtcggatgaagatatggccgccgtgaacgaatgaccggcggctttcccttatcaacaaatcatatcaaactgaaatttatggaggtaaatttatggaatttttcaatagtgcggttactactttgcagactatcgttgtgggcctcggcggtgcgctgtgtgtttggggcggcatcaaccttctggaaggttacggtcaggataacccggccagcaatgctcatgtacggtaaggaagcaagcaaccgaaaacaagagatagaccgccaacactacactattccgaaccaaagaccaaaagataagcattgtgggaaaatctaaacttttggattttcctacaatgccaactacggcggaatccctcccactccttatatctttctgtatacattgaatttgtatttagtaaaatgcagacaacaccacggatcggcttttggttggacaattccaaccaaacaccacagcagacagcagaaaacattctgaacgctaggaagccggtatgattgttacatataaggggaagaaaaatttcttttaggtacttgctttcctaaaactgatgtgatacaatgatttaatccagaaaaggagtaaaaaatatgcggcaagctattcttaaataaaactataatcaaatagtgggaacaaaggattatgatagctccttttgtaggggcttagttttttgtacccaatttaagaatacttttgccttatcaattttgacatatccccaaaaacagcaatcacaaacaggtgtatgctgtatatgtgtatgtccgcaacttataatccccagtggtaaaagtattttactgctggggatttttatgccctttggggctgtaaagggaggacaatcacatgaaaataatcaatattggaattcttgcccatgtagacgctggaaagacgaccttgacggagagcctgctatatgccagcggagccatttcagaaccggggagcgtcgaaaaagggacaacgaggacggacaccatgtttttggagcggcagcgtgggattaccattcaagcggcagtcacttccttccagtggcacagatgtaaagttaacattgtggatacgcccggccacatggattttttggcggaggtgtaccgctctttggctgttttagatggggccatcttggtgatctccgctaaagatggcgtgcaggcccagacccgtattctgttccatgccctgcggaaaatgaacattcccaccgttatctttatcaacaagatcgaccaggctggcgttgatttgcagagcgtggttcagtctgttcgggataagctctccgccgatattatcatcaagcagacggtgtcgctgtccccggaaatagtcctggaggaaaataccgacatagaagcatgggatgcggtcatcgaaaataacgatgaattattggaaaagtatatcgcaggagaaccaatcagccgggaaaaacttgcgcgggaggaacagcagcgggttcaagacgcccctgttcccagtctatcatggcagcgccaaaaatggccttggcattcaaccgttgatggatgcggtgacagggctgttccaaccgattggggaacaggggggcgccgccctatgcggcagcgttttcaaggttgagtacaccgattgcggccagcggcgtgtctatctacggttatacagcggaacgctgcgcctgcgggatacggtggccctggccgggagagaaaagctgaaaatcacagagatgcgtattccatccaaaggggaaattgttcggacagacaccgcttatcagggtgaaattgttatccttcccagcgacagcgtgaggttaaacgatgtattaggggacccaacccggctccctcgtaaaaggtggcgtgaggaccccctccccatgctgcggacgtcgattgcgccgaaaacggcagcgcaaagagaacggctgctggacgctcttacgcaacttgcggatactgacccgcttttgcgctgcgaggtggattccatcacccatgagatcattctttcttttttgggccgggtgcagttggaggttgtttccgctttgctgtcggaaaaatacaagcttgaaacagtggtaaaggaacccaccgtcatttatatggagcggccgctcaaagcagccagccacaccatccatatcgaggtgccgcccaacccgttttgggcatccatcggactgtctgttacaccactcccgcttggctccggtgtacaatacgagagccgggtttcgctgggatacttgaaccagagttttcaaa

SEQ ID NO: 3 - DNA, 2048 bp, Bifidobacterium bifidum
  source 1..2048: mol_type = genomic DNA
tttcgtggccgagcagttgcatgatgagcggtagcggcacgccctgttggtagaggtccatggcgcgggtccggcggatcaggtggcagtggacgcgttcgggcatggacgggcacgtcccgcggcgtgctctggccgccgcggttttgaggatctcgtcgatccggtccacggagagcggctggatggcgccgttcctcgtcgagtggaacaacggcctgtcgccgtcgcgcatggacggtccgggatggaattcctcgaggtaggcggccaggtgggttcgtgtcctttctcccaggggcacgacccggctcttgccgcgtttgccggtgagcgtgaccctggccggcttatccatacccacgtccgcgatggtcagtgcggcgagttcgccgatcctggcggcggtgtcgtacatgaggatcaggagcatgcggttcctgcgcgatttggcgtcgccggtgccccatgcggtcagcaacgctttggtgtgctcctccccgaggtggtcgacgggtttgcgcgcgggtggtttgacacgtatgccggccgcgtcgttgcccagcgcggtcaatgccgggtgttcgaggcccgcgtggtcgaggaacacgcgcatcgtcgtcatcctcagcatgatggtgcggtccgagtacccgcgctcggtccgcatccattcgacccaccggcccaggcgcgcccggtcgaaatgcccgaaaccgatgtggctgcgctgcgtgccttccgtggtttcgagccatcggacgtaggattccaggccgatgcggtacgcctcgacggtcttcggcgagctgccccgcaccttgggcagccagtggtgcagccagtcgcgcgcgactcgccagaagtccggttcaccggagctggcggccgttttccttgccttgctcatggttcctccgtttccgggaccacgcgttcggcgtcggcgacgaggtccgcgtatccgtccatgaaatcggggctggcgtgcacgtagtagagggtgctgtcgatgccggcgtgtcccatgtaggccgccagatagggcagcatcgccatcacgtccacgccgtcgcgagtccaccgctcgatgttcgcgaacgcgaaccggtgccggaaatcatagggcctgggccgtttgccggcttgtggccactcgagcccggcccgcgtccagacgcggcggaacaccacgccgggcatgcccggggagaccggattgccggtggaggtgacgaagaacgcgggacggtcgtctccgaagcgttcgcgggaccgttggccgcattccagcagttcggcggcgacctcgtcgcccacgggcagcctgcggctgcgaccggccttggaatcgaccacgtcgatggaacgggccttgtggtcgacgtgcccgacggcgagtctcctgacctctcgggtgcgcagcccgcagcaggccatgagcatgaagaacgcgcgagactgccacgcccacggcgacggagactccaacgttcccgcggcccgcaggaacagggcggcctcgcggtccgtcagcaggtacggcgtcggacgcggggatccggccttccactggtcggagagcacgtacgcgtcgggatcgtgggccagtcgcatccacctgccgaagtccctgatgtacgagaaccacgagcggcaacccccgggattcgcgtcgatcctatgggcgatccatcgctccacgacgccccgctccagacgcacggccccgtgttcgaggcaatgccggtcgaacgagcgcaggacctggacgcgggtggcgccatgcctgcccatggacgccttgaaacggatgtactcctccaattcgccggcgagcgggccgacgaatccgtgttccgtgggtctcatgacgatccgccttccggcacgggcagcacgcacgcgagcattcccccgcggtgcgtggccatgtagacgcgtgtggaatcggggtcggcgtggccgagcaccgcgctgatcgtcggcaacggcgtggccgcctccagcatcctcgtcgccgcgttgcgccgcaacagcctggaacc

SEQ ID NO: 4 - DNA, 541 bp, Bifidobacterium bifidum
  source 1..541: mol_type = genomic DNA
gcaggcaggaccacacgtatacggcgttgatctcataacagctgggcttgcggccgtgactgagcgccctgcacttgttccacacctcgcggatctcatgctgctcggcgatgctctcctcgcgggtgagcaccagattgccggtggatggtatcgtgtacgggctcacctcacgcggcaccttgtgttgcccggtcacgacgcgcaccagcatgccctcgacccgcctgcgcagggcggcgaggaaaccgctcatcatcttcatccgcgcgtcgggatccggctcctcgctcaccacgattcgatagcgtttcgcgctcagcatccacggactttcgcgcccgtcacgcacaccctcgacgcgatggatgatgccgactttgcccagctcgcgcagatgatagctcatggcgctggtgcttacgccgaatacctccgcaatctgcgcggcggtgcggggttcgcgtttctccgaaagctcctccaaggccgcataccgcaacgggtgcgagatgacgcgcagcacctgtcgggtccgcac

SEQ ID NO: 5 - DNA, 3001 bp, Bifidobacterium bifidum
  source 1..3001: mol_type = genomic DNA
ctatcttagatagagctgtttgaaaacagccggcgcggggtggagcagctcggtagctcgctgggctcataacccagaggtccatggttcaaatccatgccccgctaccaattgaccgtcgttcccattatcggaacggcggttttttatatactccatggcttttgctggcgttaagttctcatccagtaaagccatcaacgggacgccgaagaagtcggcagccgcgcaagtttcgtcaatggtccaatcggccttgctctgaagcctcgacgccatcgattgcggcgagagccccattgctctagcaaggtccttcttcattaaaccgctgttggacaagatcatgttcgtgttcatcgcaacaacgtcctgcctgcgcaatgtagcgctcggctgaatatctagcattgtcatgaaattcattttactacggttttagcgtagcactcggcgtgtcggctacgtcatatggttaatctttggtctagaacttcatcaaatctttagtctgaaagtttttagatgattagtcagataagaaaactcatgagagacaatcacgtcacgcagcgtgatctggcgcatgagctaggcgtctccgagcaggccatcagcgacaaattccatggccgctcaaatttcacgttgcgtgatgtgtcgcgtatagccgacttcttcgacgtctccaccgatttcgtgcttggccgtgagccgttggaggtggcgtgatggctggcgtggaacgtgtgtcggtgcatgtgagccgtctggcgcattgccctgatgtgttcttcgtcgagttctctcgtgccggttctgtggggaacctcgttgttcctctgggtcgttccgaggccgaagcgttgcgcgacgagcttggcgaagcgctgtcgggccggattacggaggccccggatgttagttgatggttttaatgatctccacgggttcagggcatccgtcccagacgatggtgaatttgatggggtaatgggctttgccgtccccgtcctccacgtgtccgtcaaagaatgtggtgccgccttgctgtcgctcctcgcgcagtttcggcagttcaatgttgaagaaatgaatgtcggacagcgcccatggtttgctgtcggttcttccgagatggttgttccatgtgttcgtgtaggttccctcgaccgcttcggcgaacacggagatgttacgcgcagggcctccgatgttggtgaggacgaaactcgccccgctttcgttgatatcaattctgaattttggcggcatgggaggcttgggagtcgccgacgttgttgtgaggaacatggcgtctatctgctcgttggatatcggtttggtctcttcgtcgtctgtgtggcggactttacgcacgacataccgaatgccggcgaacaggctaggaacgccgacgattgccaggatcactccgaggccattccaccaatctgcggacagccattcaagaatttcgttcatgtccatcaatctatccgtgccgttggaggtgtctcatgccgtatctgaagcctgaccaggccagtccggcgtcggcgatgatgtcgctgaagtccaggtgcatatattcttccttccttcgttgtttgaaaggtttggtttgtgcgattacaagcctatcgctgcggaggaaggagcctaaccgtccatccatgaatcaaggagcagtgaaatgagcgttttcgatccggaatgcgccagcaattactttcaggtgctggacatcgacccgtcggaatgcaccggcggcaatccctacggcttcaagtgccgcatcaaggtggccggaagtacgttcgggttcgatggtctggacatgggcgaccttcaggcgatgaagggcgcgatcaacaaggcgatgacgcacgctaggcgtgctcgccgtgaatgggaaggagcccaggaatgagcgtcacggtcaagcgggtggatggcaagcggtgttgcttcttcgagctgatcgtcgagacggcggacggcatgacggtgcgcgtcccgttcaacggcggcgagcttgaggacttggaaaagcagatagcgcgatgcttcgagcagtgaaacgtttcatcaagatcgttcttctgattctgctcagccccttcgtgttgttcatgctggggctggtgctcgcgatcgtccgtctgggtgatttcctcacggacgactagcaaaacgtaacggcatatggggcgtacggcgtacccctgccaccgctgagccgggttagcgaccggtaacgccaggcgcgtggctatcgcgccatttgcgagacgaaatttagctcccgaccctctcaggccgtcgattaaggcggaatcgggcgaccatagacggcttcggccgtggcctgattggggaccattcccggcggcttcggccgctcttgttatcgacggcgcggctccgaccgaaacgttctgcaagacctttggaatttgttgacggcccggccggggaatctcggccgagcgtttccatcagcagattctaggtcttgacctctcaagcgctcaccaaccgaaagctacagaaaggattgaaattgagcaaggcaacattccccgaccaactcaggacgcagatgaggatgacactcccgatgatcgacaggaacatcaggtgcagggcgaacacctcacgacagtcgttgatgaaggcgtccggattgaacgacaaccagctccaggccgctctgaaaatggcctacggagagaagggcgtgccagctcccgcccaccgttctcccaccgccggcaagatgtacgattccgagtctctgctgttgacgctggccaaatggtgcgggatgtggtcttatgtcatcgattaagccgtcattgcacgaggtgttgcactatccgaaggaatcgcgcaggatgctcatgcagggcttcgccgacgctgtggaccgcatcgcggcgagcaacgggcgcgccggcgtcgaactgtccctggtctgccgggcgctcggcgcgcc